European Patent Specification EP 3 320 773 B1, published May 10, 2023. Title: Non-human animals in which an endogenous CD3 gene has been replaced with a human CD3 gene. Applicant: CHUGAI SEIYAKU KABUSHIKI KAISHA. The sequence listing filed with the application follows.

SEQUENCE LISTING (52 sequences)

SEQ ID NO: 1 - DNA, 34 bp, Artificial
  an artificially synthesized sequence
ataacttcgtatagcatacattatacgaagttat

SEQ ID NO: 2 - DNA, 32 bp, Artificial
  an artificially synthesized sequence
taactttaaataattggcattatttaaagtta

SEQ ID NO: 3 - DNA, 34 bp, Artificial
  an artificially synthesized sequence
gaagttcctattctctagaaagtataggaacttc

SEQ ID NO: 4 - DNA, 546 bp, Homo sapiens
  CDS (1)..(546)
atggaacaggggaagggcctggctgtcctcatcctggctatcattcttcttcaaggtactttggcccagtcaatcaaaggaaaccacttggttaaggtgtatgactatcaagaagatggttcggtacttctgacttgtgatgcagaagccaaaaatatcacatggtttaaagatgggaagatgatcggcttcctaactgaagataaaaaaaaatggaatctgggaagtaatgccaaggaccctcgagggatgtatcagtgtaaaggatcacagaacaagtcaaaaccactccaagtgtattacagaatgtgtcagaactgcattgaactaaatgcagccaccatatctggctttctctttgctgaaatcgtcagcattttcgtccttgctgttggggtctacttcattgctggacaggatggagttcgccagtcgagagcttcagacaagcagactctgttgcccaatgaccagctctaccagcccctcaaggatcgagaagatgaccagtacagccaccttcaaggaaaccagttgaggaggaat

SEQ ID NO: 5 - protein, 182 aa, Homo sapiens
MEQGKGLAVLILAIILLQGTLAQSIKGNHLVKVYDYQEDGSVLLTCDAEAKNITWFKDGKMIGFLTEDKKKWNLGSNAKDPRGMYQCKGSQNKSKPLQVYYRMCQNCIELNAATISGFLFAEIVSIFVLAVGVYFIAGQDGVRQSRASDKQTLLPNDQLYQPLKDREDDQYSHLQGNQLRRN

SEQ ID NO: 6 - DNA, 513 bp, Homo sapiens
  CDS (1)..(513)
atggaacatagcacgtttctctctggcctggtactggctacccttctctcgcaagtgagccccttcaagatacctatagaggaacttgaggacagagtgtttgtgaattgcaataccagcatcacatgggtagagggaacggtgggaacactgctctcagacattacaagactggacctgggaaaacgcatcctggacccacgaggaatatataggtgtaatgggacagatatatacaaggacaaagaatctaccgtgcaagttcattatcgaatgtgccagagctgtgtggagctggatccagccaccgtggctggcatcattgtcactgatgtcattgccactctgctccttgctttgggagtcttctgctttgctggacatgagactggaaggctgtctggggctgccgacacacaagctctgttgaggaatgaccaggtctatcagcccctccgagatcgagatgatgctcagtacagccaccttggaggaaactgggctcggaacaag

SEQ ID NO: 7 - protein, 171 aa, Homo sapiens
MEHSTFLSGLVLATLLSQVSPFKIPIEELEDRVFVNCNTSITWVEGTVGTLLSDITRLDLGKRILDPRGIYRCNGTDIYKDKESTVQVHYRMCQSCVELDPATVAGIIVTDVIATLLLALGVFCFAGHETGRLSGAADTQALLRNDQVYQPLRDRDDAQYSHLGGNWARNK

SEQ ID NO: 8 - DNA, 621 bp, Homo sapiens
  CDS (1)..(621)
atgcagtcgggcactcactggagagttctgggcctctgcctcttatcagttggcgtttgggggcaagatggtaatgaagaaatgggtggtattacacagacaccatataaagtctccatctctggaaccacagtaatattgacatgccctcagtatcctggatctgaaatactatggcaacacaatgataaaaacataggcggtgatgaggatgataaaaacataggcagtgatgaggatcacctgtcactgaaggaattttcagaattggagcaaagtggttattatgtctgctaccccagaggaagcaaaccagaagatgcgaacttttatctctacctgagggcaagagtgtgtgagaactgcatggagatggatgtgatgtcggtggccacaattgtcatagtggacatctgcatcactgggggcttgctgctgctggtttactactggagcaagaatagaaaggccaaggccaagcctgtgacacgaggagcgggtgctggcggcaggcaaaggggacaaaacaaggagaggccaccacctgttcccaacccagactatgagcccatccggaaaggccagcgggacctgtattctggcctgaatcagagacgcatc

SEQ ID NO: 9 - protein, 207 aa, Homo sapiens
MQSGTHWRVLGLCLLSVGVWGQDGNEEMGGITQTPYKVSISGTTVILTCPQYPGSEILWQHNDKNIGGDEDDKNIGSDEDHLSLKEFSELEQSGYYVCYPRGSKPEDANFYLYLRARVCENCMEMDVMSVATIVIVDICITGGLLLLVYYWSKNRKAKAKPVTRGAGAGGRQRGQNKERPPPVPNPDYEPIRKGQRDLYSGLNQRRI

SEQ ID NO: 10 - protein, 4 aa, Artificial
  an artificially synthesized sequence
GGGS

SEQ ID NO: 11 - protein, 4 aa, Artificial
  an artificially synthesized sequence
SGGG

SEQ ID NO: 12 - protein, 5 aa, Artificial
  an artificially synthesized sequence
GGGGS

SEQ ID NO: 13 - protein, 5 aa, Artificial
  an artificially synthesized sequence
SGGGG

SEQ ID NO: 14 - protein, 6 aa, Artificial
  an artificially synthesized sequence
GGGGGS

SEQ ID NO: 15 - protein, 6 aa, Artificial
  an artificially synthesized sequence
SGGGGG

SEQ ID NO: 16 - protein, 7 aa, Artificial
  an artificially synthesized sequence
GGGGGGS

SEQ ID NO: 17 - protein, 7 aa, Artificial
  an artificially synthesized sequence
SGGGGGG

SEQ ID NO: 18 - DNA, 20 bp, Artificial
  an artificially synthesized sequence
tatcagagcttggttgacgg

SEQ ID NO: 19 - DNA, 32 bp, Artificial
  an artificially synthesized sequence
actcgttgtggcttagaagcagtaacaatacc

SEQ ID NO: 20 - DNA, 30 bp, Artificial
  an artificially synthesized sequence
actgtaatcctagtacttaggaggctgagg

SEQ ID NO: 21 - DNA, 26 bp, Artificial
  an artificially synthesized sequence
aatccatcttgttcaatggccgatcc

SEQ ID NO: 22 - DNA, 30 bp, Artificial
  an artificially synthesized sequence
tagcagccttcagatgaagaggtaggactc

SEQ ID NO: 23 - DNA, 28 bp, Artificial
  an artificially synthesized sequence
ttgatgtgccacctcactgctgcactgg

SEQ ID NO: 24 - DNA, 24 bp, Artificial
  an artificially synthesized sequence
aactgacaatgggacatcagctga

SEQ ID NO: 25 - DNA, 24 bp, Artificial
  an artificially synthesized sequence
atgggactgttactttactaagat

SEQ ID NO: 26 - DNA, 28 bp, Artificial
  an artificially synthesized sequence
aagaaatgggtggtattacacagacacc

SEQ ID NO: 27 - DNA, 31 bp, Artificial
  an artificially synthesized sequence
tgggccagcgggaggcagtgttctccagagg

SEQ ID NO: 28 - DNA, 29 bp, Artificial
  an artificially synthesized sequence
tagttcggtgacctggctttatctactgg

SEQ ID NO: 29 - DNA, 31 bp, Artificial
  an artificially synthesized sequence
atggctgcttctagaagccaccagtctcagg

SEQ ID NO: 30 - DNA, 26 bp, Artificial
  an artificially synthesized sequence
tgctccacgcttttgccggaggacag

SEQ ID NO: 31 - DNA, 25 bp, Artificial
  an artificially synthesized sequence
taggaggagaacacctggactactc

SEQ ID NO: 32 - DNA, 28 bp, Artificial
  an artificially synthesized sequence
agcattctgagaggatgcggtggaacac

SEQ ID NO: 33 - DNA, 29 bp, Artificial
  an artificially synthesized sequence
tgctcggagggctggatctgggtccacag

SEQ ID NO: 34 - DNA, 29 bp, Artificial
  an artificially synthesized sequence
tcatcctgtggcttgcctctatttgttgc

SEQ ID NO: 35 - DNA, 29 bp, Artificial
  an artificially synthesized sequence
ttgctatggcactttgagaaacctccatc

SEQ ID NO: 36 - DNA, 26 bp, Artificial
  an artificially synthesized sequence
aatacttctactggagaagcaaagag

SEQ ID NO: 37 - DNA, 27 bp, Artificial
  an artificially synthesized sequence
tagttgcatttagaggacttattatgc

SEQ ID NO: 38 - DNA, 360 bp, Artificial
  an artificially synthesized sequence
  CDS (1)..(360)
gaagtgcagctggtcgagagcgggggggggctggtgcagccaggaggatctctgaggctgagttgcgccgcttcaggcttcaacatcaaggacacttacattcactgggtgcgacaggcaccagggaaaggactggagtgggtcgcccggatctatcccacaaatggatacactcggtatgccgactccgtgaagggcagattcaccattagcgccgatacctccaaaaacacagcttacctgcagatgaacagcctgagggctgaagatacagcagtgtactattgctctcgctggggaggcgacggcttttacgcaatggattattggggccaggggactctggtgaccgtcagctcc

SEQ ID NO: 39 - protein, 120 aa, Artificial [sequence omitted]

SEQ ID NO: 40 - DNA, 321 bp, Artificial
  an artificially synthesized sequence
  CDS (1)..(321)
gacattcagatgactcagagcccttcaagcctgagtgcttcagtcggggacagggtgacaatcacttgccgcgcaagccaggatgtcaacaccgctgtggcatggtaccagcagaagccaggcaaagcacccaagctgctgatctacagcgcctccttcctgtattccggggtgccatctcggttttctggcagtagatcagggaccgacttcaccctgacaatcagctccctgcagcccgaagattttgccacatactattgccagcagcactacaccacaccccctacattcgggcagggaactaaagtggagattaag

SEQ ID NO: 41 - protein, 107 aa, Artificial [sequence omitted]

SEQ ID NO: 42 - DNA, 321 bp, Artificial
  an artificially synthesized sequence
  CDS (1)..(321)
gatattcagatgactcagagcccttcttcactgagtgcatcagtgggcgaccgagtcaccatcacatgccgggccagccaggatattagaaactacctgaattggtatcagcagaagcctggcaaagctccaaagctgctgatctactatacctctaggctggagagtggagtgccatcacgcttcagcggatccggatctgggaccgactacactctgaccattagctccctgcagccagaagatttcgccacatactattgtcagcagggaaacactctgccctggacctttggacagggcaccaaagtggagatcaag

SEQ ID NO: 43 - protein, 107 aa, Artificial [sequence omitted]

SEQ ID NO: 44 - DNA, 366 bp, Artificial
  an artificially synthesized sequence
  CDS (1)..(366)
gaggtgcagctggtcgaatccggaggaggactggtgcagccaggaggaagcctgcgactgtcctgcgccgctagcggatactcctttacaggctatactatgaattgggtgcgacaggctcccgggaaaggactggagtgggtggcactgatcaacccttacaagggcgtcagtacctataatcagaagttcaaagaccggttcaccatttctgtggataagagtaaaaacaccgcttacctgcagatgaatagcctgagagcagaggacacagccgtgtactattgcgcaaggagtggctactatggggactcagattggtatttcgacgtgtggggacaggggaccctggtgacagtctctagt

SEQ ID NO: 45 - protein, 122 aa, Artificial [sequence omitted]

SEQ ID NO: 46 - protein, 118 aa, Artificial Sequence
  an artificially synthesized sequence
QVQLVESGGGVVQPGRSLRLSCAASGFTFSSYTMHWVRQAPGKGLEWVTFISYDGNNKYYADSVKGRFTISRDNSKNTLYLQMNSLRAEDTAIYYCARTGWLGPFDYWGQGTLVTVSS

SEQ ID NO: 47 - protein, 108 aa, Artificial Sequence
  an artificially synthesized sequence
EIVLTQSPGTLSLSPGERATLSCRASQSVGSSYLAWYQQKPGQAPRLLIYGAFSRATGIPDRFSGSGSGTDFTLTISRLEPEDFAVYYCQQYGSSPWTFGQGTKVEIK

SEQ ID NO: 48 - protein, 324 aa, Artificial Sequence
  an artificially synthesized sequence
AKTTPPSVYPLAPGSAAQTNSMVTLGCLVKGYFPEPVTVTWNSGSLSSGVHTFPAVLQSDLYTLSSSVTVPSSTWPSETVTCNVAHPASSTKVDKKIVPRDCGCKPCICTVKEVSKVFIFPPKPKDVLTITLTPKVTCVVVDISKDDPEVQFSWFVDDVEVHTAQTQPREEQFNSTFRSVSELPIMHQDWLNGKEFKCRVNSAAFPAPIEKTISKTKGRPKAPQVYTIPPPKEQMAKDKVSLTCMITDFFPEDITVEWQWNGQPAENYKNTQPIMDTDGSYFVYSELNVQKSNWEAGNTFTCSVLHEGLHNHHTEKSLSHSPGK

SEQ ID NO: 49 - protein, 107 aa, Artificial Sequence
  an artificially synthesized sequence
RADAAPTVSIFPPSSEQLTSGGASVVCFLNNFYPKDINVKWKIDGSERQNGVLNSWTDQDSKDSTYSMSSTLTLTKDEYERHNSYTCEATHKTSTSPIVKSFNRNEC

SEQ ID NO: 50 - protein, 122 aa, Artificial Sequence
  an artificially synthesized sequence
QVQLVESGGGVVQPGGSLRLSCAASGFTFSNAWMHWVRQAPGKGLEWVAQIKDKSQNYATYVAESVKGRFTISRADSKNSIYLQMNSLKTEDTAVYYCRYVHYAAGYGVDIWGQGTTVTVSS

SEQ ID NO: 51 - protein, 112 aa, Artificial Sequence
  an artificially synthesized sequence
DIVMTQSPLSLPVTPGEPASISCRSSQPLVHSNRNTYLHWYQQKPGQAPRLLIYKVSNRFSGVPDRFSGSGSGTDFTLKISRVEAEDVGVYYCGQGTQVPYTFGQGTKLEIK

SEQ ID NO: 52 - protein, 324 aa, Artificial Sequence
  an artificially synthesized sequence
AKTTPPSVYPLAPGSAAQTNSMVTLGCLVKGYFPEPVTVTWNSGSLSSGVHTFPAVLQSDLYTLSSSVTVPSSTWPSETVTCNVAHPASSTKVDKKIVPRDCGCKPCICTVKEVSKVFIFPPKPKDVLTITLTPKVTCVVVDISKDDPEVQFSWFVDDVEVHTAQTQPREEQFNSTFRSVSELPIMHQDWLNGKEFKCRVNSAAFPAPIEKTISKTKGRPKAPQVYTIPPPKEQMAKDKVSLTCMITDFFPEDITVEWQWNGQPAENYKNTQPIMRTDGSYFVYSKLNVQKSNWEAGNTFTCSVLHEGLHNHHTEKSLSHSPGK